European Patent Specification EP 3 411 409 B1, published October 8, 2025. Title: METHODS AND COMPOSITIONS FOR ENHANCING THE POTENCY OF SUPERANTIGEN MEDIATED CANCER IMMUNOTHERAPY. Applicant: NeoTX Ltd. The sequence listing filed with the application follows.

SEQUENCE LISTING (10 sequences)

SEQ ID NO: 1 - protein, 233 aa, Staphylococcus sp
SEKSEEINEKDLRKKSELQRNALSNLRQIYYYNEKAITENKESDDQFLENTLLFKGFFTGHPWYNDLLVDLGSKDATNKYKGKKVDLYGAYYGYQCAGGTPNKTACMYGGVTLHDNNRLTEEKKVPINLWIDGKQTTVPIDKVKTSKKEVTVQELDLQARHYLHGKFGLYNSDSFGGKVQRGLIVFHSSEGSTVSYDLFDAQGQYPDTLLRIYRDNKTINSENLHIDLYLYTT

SEQ ID NO: 2 - protein, 233 aa, Staphylococcus sp
SEKSEEINEKDLRKKSELQGTALGNLKQIYYYNEKAKTENKESHDQFLQHTILFKGFFTDHSWYNDLLVDFDSKDIVDKYKGKKVDLYGAYYGYQCAGGTPNKTACMYGGVTLHDNNRLTEEKKVPINLWLDGKQNTVPLETVKTNKKNVTVQELDLQARRYLQEKYNLYNSDVFDGKVQRGLIVFHTSTEPSVNYDLFGAQGQYSNTLLRIYRDNKTINSENMHIDIYLYTS

SEQ ID NO: 3 - protein, 233 aa, Artificial Sequence
  Mutated Protein
SEKSEEINEKDLRKKSELQGTALGNLKQIYYYNSKAITSSEKSADQFLTNTLLFKGFFTGHPWYNDLLVDLGSTAATSEYEGSSVDLYGAYYGYQCAGGTPNKTACMYGGVTLHDNNRLTEEKKVPINLWIDGKQTTVPIDKVKTSKKEVTVQELDLQARHYLHGKFGLYNSDSFGGKVQRGLIVFHSSEGSTVSYDLFDAQGQYPDTLLRIYRDNTTISSTSLSISLYLYTT

SEQ ID NO: 4 - protein, 233 aa, Artificial Sequence
  Mutated Protein
SEKSEEINEKDLRKKSELQGTALGNLKQIYYYNEKAKTENKESHDQFLQHTILFKGFFTDHSWYNDLLVDFDSKDIVDKYKGKKVDLYGAYYGYQCAGGTPNKTACMYGGVTLHDNNRLTEEKKVPINLWLDGKQNTVPLETVKTNKKNVTVQELDLQARRYLQEKYNLYNSDVFDGKVQRGLIVFHTSTEPSVNYDLFGAQGQYSNTLLRIYRDNKTINSENMHIAIYLYTS

SEQ ID NO: 5 - protein, 679 aa, Artificial Sequence
  Conjugated Protein
  MISC_FEATURE (460)..(679): Light Chain
QVQLQQPGAELVRPGASVKLSCKASGYTFTNYWINWVKQRPGQGLEWIGNIYPSYIYTNYNQEFKDKVTLTVDESSSTAYMQLSSPTSEDSAVYYCTRSPYGYDEYGLDYWGQGTSVTVSSAKTTPPSVYPLAPGSAAQTNSMVTLGCLVKGYFPEPVTVTWNSGSLSSGVHTFPAVLQSDLYTLSSSVTVPSSTWPSETVTCNVAHPASSTKVDKKIVPRDSGGPSEKSEEINEKDLRKKSELQGTALGNLKQIYYYNEKAKTENKESHDQFLQHTILFKGFFTDHSWYNDLLVDFDSKDIVDKYKGKKVDLYGAYYGYQCAGGTPNKTACMYGGVTLHDNNRLTEEKKVPINLWLDGKQNTVPLETVKTNKKNVTVQELDLQARRYLQEKYNLYNSDVFDGKVQRGLIVFHTSTEPSVNYDLFGAQGQYSNTLLRIYRDNKTINSENMHIDIYLYTSDIVMTQSPSSLTVTAGEKVTMNCKSSQSLLNSRNQKNYLTWYQQKPGQPPKLLIYWASTRESGVPDRFTGSGSGTDFTLTISSVQAEDLAVYYCQNDYVYPLTFGAGTKLELKRADAAPTVSIFPPSSEQLTSGGASVVCFLNNFYPKDINVKWKIDGSERQNGVLNSWTDQDSKDSTYSMSSTLTLTKDEYERHNSYTCEATHKTSTSPIVKSFNRNES

SEQ ID NO: 6 - protein, 672 aa, Artificial Sequence
  Mutated and Conjugated Protein
  MISC_FEATURE (459)..(672): Light Chain
EVQLQQSGPDLVKPGASVKISCKASGYSFTGYYMHWVKQSHGKSLEWIGRINPNNGVTLYNQKFKDKAILTVDKSSTTAYMELRSLTSEDSAVYYCARSTMITNYVMDYWGQVTSVTVSSAKTTPPSVYPLAPGSAAQTNSMVTLGCLVKGYFPEPVTVTWNSGSLSSGVHTFPAVLQSDLYTLSSSVTVPSSTWPSETVTCNVAHPASSTKVDKKIVPRDSGGPSEKSEEINEKDLRKKSELQGTALGNLKQIYYYNEKAKTENKESHDQFLQHTILFKGFFTDHSWYNDLLVDFDSKDIVDKYKGKKVDLYGAYYGYQCAGGTPNKTACMYGGVTLHDNNRLTEEKKVPINLWLDGKQNTVPLETVKTNKKNVTVQELDLQARRYLQEKYNLYNSDVFDGKVQRGLIVFHTSTEPSVNYDLFGAQGQYSNTLLRIYRDNKTINSENMHIAIYLYTSSIVMTQTPTSLLVSAGDRVTITCKASQSVSNDVAWYQQKPGQSPKLLISYTSSRYAGVPDRFSGSGSGTDFTLTISSVQAEDLAVYFCQQDYNSPPTFGGGTKLEIKRADAAPTVSIFPPSSEQLTSGGASVVCFLNNFYPKDINVKWKIDGSERQNGVLNSWTDQDSKDSTYSMSSTLTLTKDEYERHNSYTCEATHKTSTSPIVKSFNRNES

SEQ ID NO: 7 - protein, 672 aa, Artificial Sequence
  Mutated and Conjugated Protein
  MISC_FEATURE (459)..(672): Light Chain
EVQLQQSGPDLVKPGASVKISCKASGYSFTGYYMHWVKQSPGKGLEWIGRINPNNGVTLYNQKFKDKATLTVDKSSTTAYMELRSLTSEDSAVYYCARSTMITNYVMDYWGQGTSVTVSSAKTTPPSVYPLAPGSAAQTNSMVTLGCLVKGYFPEPVTVTWNSGSLSSGVHTFPAVLQSDLYTLSSSVTVPSSTWPSETVTCNVAHPASSTKVDKKIVPRDSGGPSEKSEEINEKDLRKKSELQGTALGNLKQIYYYNSKAITSSEKSADQFLTNTLLFKGFFTGHPWYNDLLVDLGSTAATSEYEGSSVDLYGAYYGYQCAGGTPNKTACMYGGVTLHDNNRLTEEKKVPINLWIDGKQTTVPIDKVKTSKKEVTVQELDLQARHYLHGKFGLYNSDSFGGKVQRGLIVFHSSEGSTVSYDLFDAQGQYPDTLLRIYRDNTTISSTSLSISLYLYTTSIVMTQTPTSLLVSAGDRVTITCKASQSVSNDVAWYQQKPGQSPKLLISYTSSRYAGVPDRFSGSGYGTDFTLTISSVQAEDAAVYFCQQDYNSPPTFGGGTKLEIKRADAAPTVSIFPPSSEQLTSGGASVVCFLNNFYPKDINVKWKIDGSERQNGVLNSWTDQDSKDSTYSMSSTLTLTKDEYERHNSYTCEATHKTSTSPIVKSFNRNES

SEQ ID NO: 8 - protein, 458 aa, Artificial Sequence
  Synthetic polypeptide
EVQLQQSGPDLVKPGASVKISCKASGYSFTGYYMHWVKQSPGKGLEWIGRINPNNGVTLYNQKFKDKATLTVDKSSTTAYMELRSLTSEDSAVYYCARSTMITNYVMDYWGQGTSVTVSSAKTTPPSVYPLAPGSAAQTNSMVTLGCLVKGYFPEPVTVTWNSGSLSSGVHTFPAVLQSDLYTLSSSVTVPSSTWPSETVTCNVAHPASSTKVDKKIVPRDSGGPSEKSEEINEKDLRKKSELQGTALGNLKQIYYYNSKAITSSEKSADQFLTNTLLFKGFFTGHPWYNDLLVDLGSTAATSEYEGSSVDLYGAYYGYQCAGGTPNKTACMYGGVTLHDNNRLTEEKKVPINLWIDGKQTTVPIDKVKTSKKEVTVQELDLQARHYLHGKFGLYNSDSFGGKVQRGLIVFHSSEGSTVSYDLFDAQGQYPDTLLRIYRDNTTISSTSLSISLYLYTT

SEQ ID NO: 9 - protein, 214 aa, Artificial Sequence
  Synthetic polypeptide
SIVMTQTPTSLLVSAGDRVTITCKASQSVSNDVAWYQQKPGQSPKLLISYTSSRYAGVPDRFSGSGYGTDFTLTISSVQAEDAAVYFCQQDYNSPPTFGGGTKLEIKRADAAPTVSIFPPSSEQLTSGGASVVCFLNNFYPKDINVKWKIDGSERQNGVLNSWTDQDSKDSTYSMSSTLTLTKDEYERHNSYTCEATHKTSTSPIVKSFNRNES

SEQ ID NO: 10 - protein, 233 aa, Artificial Sequence
  Mutated Protein
SEKSEEINEKDLRKKSELQGTALGNLKQIYYYNEKAITENKESDDQFLENTLLFKGFFTGHPWYNDLLVDLGSKDATNKYKGKKVDLYGAYYGYQCAGGTPNKTACMYGGVTLHDNNRLTEEKKVPINLWIDGKQTTVPIDKVKTSKKEVTVQELDLQARHYLHGKFGLYNSDSFGGKVQRGLIVFHSSEGSTVSYDLFDAQGQYPDTLLRIYRDNKTINSENLHIALYLYTT